European Patent Application EP 4 353 253 A1, published April 17, 2024. Title: PURIFYING TCR-MODIFIED T CELLS USING TCR-SPECIFIC CAR-NK CELLS. Applicant: Charité - Universitätsmedizin Berlin. The sequence listing filed with the application follows.

SEQUENCE LISTING (53 sequences)

SEQ ID NO: 1 - DNA, 399 bp, synthetic construct
  source 1..399: mol_type = other DNA
accgtttttctggacaaccccaaagtaccccgtctccctggctttagccacctctccatcctcttgctttctttgcctggacaccccgttctcctgtggattcgggtcacctctcactcctttcatttgggcagctcccctaccccccttacctctctagtctgtgctagctcttccagccccctgtcatggcatcttccaggggtccgagagctcagctagtcttcttcctccaacccgggcccctatgtccacttcaggacagcatgtttgctgcctccagggatcctgtgtccccgagctgggaccaccttatattcccagggccggttaatgtggctctggttctgggtacttttatctgtcccctccaccccacagtggggccactagggacag

SEQ ID NO: 2 - DNA, 626 bp, synthetic construct
  source 1..626: mol_type = other DNA
cattgattattgagtagttattaatagtaatcaattacggggtcattagttcatagcccatatatggagttccgcgttacataacttacggtaaatggcccgcctggctgaccgcccaacgacccccgcccattgacgtcaataatgacgtatgttcccatagtaacgccaatagggactttccattgacgtcaatgggtggagtatttacggtaaactgcccacttggcagtacatcaagtgtatcatatgccaagtacgccccctattgacgtcaatgacggtaaatggcccgcctggcattatgcccagtacatgaccttatgggactttcctacttggcagtacatctacgtattagtcatcgctattaccatggtgatgcggttttggcagtacatcaatgggcgtggatagcggtttgactcacggggatttccaagtctccaccccattgacgtcaatgggagtttgttttggcaccaaaatcaacgggactttccaaaatgtcgtaacaactccgccccattgacgcaaatgggcggtaggcgtgtacggtgggaggtctatataagcagagctggtttagtgaaccgtcagatccgctagcgctaccggtcgccacc

SEQ ID NO: 3 - DNA, 63 bp, synthetic construct
  source 1..63: mol_type = other DNA
atggctcttcctgtgactgcccttctgctgcccctggctctcctgctccatgctgcccggcca

SEQ ID NO: 4 - DNA, 30 bp, synthetic construct
  source 1..30: mol_type = other DNA
gagcaaaaacttatctctgaagaggacctc

SEQ ID NO: 5 - DNA, 738 bp, synthetic construct
  source 1..738: mol_type = other DNA
gaagtacagctgcagcaaagtggtcccgaattggtgaaacccggtgcatccgtgaaaatgagttgcaaagcatctggctacaaatttacctcctatgtcatgcattgggtgaagcaaaagcccggacaaggcttggagtggatcggctatatcaacccatataacgacgtaacgaaatacaatgaaaaatttaaaggcaaggcgactctgacctcagacaaatctagctctactgcttacatggagctctccagtctgacgagcgaagacagcgccgttcattactgtgcacgaggttcttattatgattacgatggttttgtctattggggacaaggaacgcttgtcactgtatctgctggaggtggtggatcaggaggtggaggttccggaggtggaggaagtggcggtggaggtagccaaattgtgctgacacagagcccggcaatcatgagcgcatctcccggagaaaaggtcaccatgacatgttctgccacctcttctgtctcttacatgcactggtatcagcagaaatcaggcacaagtcctaagagatggatatacgacacaagcaaactggcgagcggagtgcctgctcgcttctccggcagtggaagcgggactagctatagccttaccatcagcagcatggaggccgaagacgccgcaacctactattgtcaacagtggtccagtaaccctctgacttttggagccggaacaaagctggaactcaag

SEQ ID NO: 6 - DNA, 738 bp, synthetic construct
  source 1..738: mol_type = other DNA
caagtgcagctccaacagtctggcgctgagcttgccagaccaggcgcctcagtgaaaatgagttgcaaggccagcggttacaccttcacccgctatacaatgcactgggtgaagcaaagaccgggccagggcctcgaatggatcggctacataaatccatccagggggtacaccaattacaaccagaaattcaaagataaagcaaccctcactaccgacaagagttcaagcacggcttacatgcaactttccagtctgacgtcagaggactccgctgtttactactgcgcacgctactatgatgatcattactcactggattattggggacagggaactacgcttaccgtgtccagcggaggtggtggatcaggaggtggaggttccggaggtggaggaagtggcggtggaggtagcgacatcgtactgactcaatcacccgccattatgagtgcatcaccaggcgagaaagttaccatgacttgttcagcctcatcatctgttagctacatgaattggtatcaacagaagtctgggacctccccaaagagatggatatatgatacctccaaacttgcctctggggtgcctgcacactttagaggaagcggcagcggaaccagctactctctgaccatcagtggaatggaagctgaggacgcagccacctactactgccagcagtggagctctaatccatttacattcggctctggcaccaagcttgaaataaaccgc

SEQ ID NO: 7 - DNA, 321 bp, synthetic construct
  source 1..321: mol_type = other DNA
atagaagtaatgtatccccctccctacttggacaacgagaaatctaacggcacaatcatacacgttaagggcaagcatctgtgtccctcccctcttttccccggaccgtctaagccattttgggtcctcgtggtggtcgggggtgtgctggcctgctacagcttgctggtcacagtggccttcatcatcttctgggtgcgctccaagaggagccggctgcttcacagtgattacatgaacatgacccccaggaggccaggacccaccaggaagcactaccagccctacgctcccccgcgggactttgctgcttaccgcagc

SEQ ID NO: 8 - DNA, 237 bp, synthetic construct
  source 1..237: mol_type = other DNA
ttcgtgccagttttcttacccgcgaagccgaccacaacaccagcaccgcgcccaccaacaccagctcccacaatagcctcgcagccgctctcactgcgcccggaggcttgtaggcccgctgccggtggagcagttcatacgcgaggacttgatttcgcctgtgacatatatatttgggcacctctcgccggaacctgtggggtcttgctgctgtctctcgttataacgctttattgc

SEQ ID NO: 9 - DNA, 126 bp, synthetic construct
  source 1..126: mol_type = other DNA
aaacggggcagaaagaaactcctgtatatattcaaacaaccatttatgagaccagtacaaactactcaagaggaagatggctgtagctgccgatttccagaagaagaagaaggaggatgtgaactg

SEQ ID NO: 10 - DNA, 339 bp, synthetic construct
  source 1..339: mol_type = other DNA
agggtcaaattttctagatctgcagatgcgccggcctatcaacaaggccagaaccagctctataacgagctcaatctaggacgaagagaggagtacgatgttttggacaagagacgtggccgggaccctgagatggggggaaagccgagaaggaagaaccctcaggaaggcctgtacaatgaactgcagaaagataagatggcggaggcctacagtgagattgggatgaaaggcgagcgccggaggggcaaggggcacgatggcctttaccagggtctcagtacagccaccaaggacacctacgacgcccttcacatgcaggccctgccccctcgctaa

SEQ ID NO: 11 - DNA, 46 bp, synthetic construct
  source 1..46: mol_type = other DNA
agatctcgagtctagctcgagggcgcgccccgctgatcagcctcga

SEQ ID NO: 12 - DNA, 225 bp, synthetic construct
  source 1..225: mol_type = other DNA
ctgtgccttctagttgccagccatctgttgtttgcccctcccccgtgccttccttgaccctggaaggtgccactcccactgtcctttcctaataaaatgaggaaattgcatcgcattgtctgagtaggtgtcattctattctggggggtggggtggggcaggacagcaagggggaggattgggaagacaatagcaggcatgctggggatgcggtgggctctatgg

SEQ ID NO: 13 - DNA, 400 bp, synthetic construct
  source 1..400: mol_type = other DNA
gattggtgacagaaaagccccatccttaggcctcctccttcctagtctcctgatattgggtctaacccccacctcctgttaggcagattccttatctggtgacacacccccatttcctggagccatctctctccttgccagaacctctaaggtttgcttacgatggagccagagaggatcctgggagggagagcttggcagggggtgggagggaagggggggatgcgtgacctgcccggttctcagtggccaccctgcgctaccctctcccagaacctgagctgctctgacgcggccgtctggtgcgtttcactgatcctggtgctgcagcttccttacacttcccaagaggagaagcagtttggaaaaacaaaatcagaataagttggtcctgagttct

SEQ ID NO: 14 - DNA, 3187 bp, synthetic construct
  source 1..3187: mol_type = other DNA
accgtttttctggacaaccccaaagtaccccgtctccctggctttagccacctctccatcctcttgctttctttgcctggacaccccgttctcctgtggattcgggtcacctctcactcctttcatttgggcagctcccctaccccccttacctctctagtctgtgctagctcttccagccccctgtcatggcatcttccaggggtccgagagctcagctagtcttcttcctccaacccgggcccctatgtccacttcaggacagcatgtttgctgcctccagggatcctgtgtccccgagctgggaccaccttatattcccagggccggttaatgtggctctggttctgggtacttttatctgtcccctccaccccacagtggggccactagggacagcattgattattgagtagttattaatagtaatcaattacggggtcattagttcatagcccatatatggagttccgcgttacataacttacggtaaatggcccgcctggctgaccgcccaacgacccccgcccattgacgtcaataatgacgtatgttcccatagtaacgccaatagggactttccattgacgtcaatgggtggagtatttacggtaaactgcccacttggcagtacatcaagtgtatcatatgccaagtacgccccctattgacgtcaatgacggtaaatggcccgcctggcattatgcccagtacatgaccttatgggactttcctacttggcagtacatctacgtattagtcatcgctattaccatggtgatgcggttttggcagtacatcaatgggcgtggatagcggtttgactcacggggatttccaagtctccaccccattgacgtcaatgggagtttgttttggcaccaaaatcaacgggactttccaaaatgtcgtaacaactccgccccattgacgcaaatgggcggtaggcgtgtacggtgggaggtctatataagcagagctggtttagtgaaccgtcagatccgctagcgctaccggtcgccaccatggctcttcctgtgactgcccttctgctgcccctggctctcctgctccatgctgcccggccagagcaaaaacttatctctgaagaggacctcgaagtacagctgcagcaaagtggtcccgaattggtgaaacccggtgcatccgtgaaaatgagttgcaaagcatctggctacaaatttacctcctatgtcatgcattgggtgaagcaaaagcccggacaaggcttggagtggatcggctatatcaacccatataacgacgtaacgaaatacaatgaaaaatttaaaggcaaggcgactctgacctcagacaaatctagctctactgcttacatggagctctccagtctgacgagcgaagacagcgccgttcattactgtgcacgaggttcttattatgattacgatggttttgtctattggggacaaggaacgcttgtcactgtatctgctggaggtggtggatcaggaggtggaggttccggaggtggaggaagtggcggtggaggtagccaaattgtgctgacacagagcccggcaatcatgagcgcatctcccggagaaaaggtcaccatgacatgttctgccacctcttctgtctcttacatgcactggtatcagcagaaatcaggcacaagtcctaagagatggatatacgacacaagcaaactggcgagcggagtgcctgctcgcttctccggcagtggaagcgggactagctatagccttaccatcagcagcatggaggccgaagacgccgcaacctactattgtcaacagtggtccagtaaccctctgacttttggagccggaacaaagctggaactcaagatagaagtaatgtatccccctccctacttggacaacgagaaatctaacggcacaatcatacacgttaagggcaagcatctgtgtccctcccctcttttccccggaccgtctaagccattttgggtcctcgtggtggtcgggggtgtgctggcctgctacagcttgctggtcacagtggccttcatcatcttctgggtgcgctccaagaggagccggctgcttcacagtgattacatgaacatgacccccaggaggccaggacccaccaggaagcactaccagccctacgctcccccgcgggactttgctgcttaccgcagcagggtcaaattttctagatctgcagatgcgccggcctatcaacaaggccagaaccagctctataacgagctcaatctaggacgaagagaggagtacgatgttttggacaagagacgtggccgggaccctgagatggggggaaagccgagaaggaagaaccctcaggaaggcctgtacaatgaactgcagaaagataagatggcggaggcctacagtgagattgggatgaaaggcgagcgccggaggggcaaggggcacgatggcctttaccagggtctcagtacagccaccaaggacacctacgacgcccttcacatgcaggccctgccccctcgctaaagatctcgagtctagctcgagggcgcgccccgctgatcagcctcgactgtgccttctagttgccagccatctgttgtttgcccctcccccgtgccttccttgaccctggaaggtgccactcccactgtcctttcctaataaaatgaggaaattgcatcgcattgtctgagtaggtgtcattctattctggggggtggggtggggcaggacagcaagggggaggattgggaagacaatagcaggcatgctggggatgcggtgggctctatgggattggtgacagaaaagccccatccttaggcctcctccttcctagtctcctgatattgggtctaacccccacctcctgttaggcagattccttatctggtgacacacccccatttcctggagccatctctctccttgccagaacctctaaggtttgcttacgatggagccagagaggatcctgggagggagagcttggcagggggtgggagggaagggggggatgcgtgacctgcccggttctcagtggccaccctgcgctaccctctcccagaacctgagctgctctgacgcggccgtctggtgcgtttcactgatcctggtgctgcagcttccttacacttcccaagaggagaagcagtttggaaaaacaaaatcagaataagttggtcctgagttct

SEQ ID NO: 15 - DNA, 3187 bp, synthetic construct
  source 1..3187: mol_type = other DNA
accgtttttctggacaaccccaaagtaccccgtctccctggctttagccacctctccatcctcttgctttctttgcctggacaccccgttctcctgtggattcgggtcacctctcactcctttcatttgggcagctcccctaccccccttacctctctagtctgtgctagctcttccagccccctgtcatggcatcttccaggggtccgagagctcagctagtcttcttcctccaacccgggcccctatgtccacttcaggacagcatgtttgctgcctccagggatcctgtgtccccgagctgggaccaccttatattcccagggccggttaatgtggctctggttctgggtacttttatctgtcccctccaccccacagtggggccactagggacagcattgattattgagtagttattaatagtaatcaattacggggtcattagttcatagcccatatatggagttccgcgttacataacttacggtaaatggcccgcctggctgaccgcccaacgacccccgcccattgacgtcaataatgacgtatgttcccatagtaacgccaatagggactttccattgacgtcaatgggtggagtatttacggtaaactgcccacttggcagtacatcaagtgtatcatatgccaagtacgccccctattgacgtcaatgacggtaaatggcccgcctggcattatgcccagtacatgaccttatgggactttcctacttggcagtacatctacgtattagtcatcgctattaccatggtgatgcggttttggcagtacatcaatgggcgtggatagcggtttgactcacggggatttccaagtctccaccccattgacgtcaatgggagtttgttttggcaccaaaatcaacgggactttccaaaatgtcgtaacaactccgccccattgacgcaaatgggcggtaggcgtgtacggtgggaggtctatataagcagagctggtttagtgaaccgtcagatccgctagcgctaccggtcgccaccatggctcttcctgtgactgcccttctgctgcccctggctctcctgctccatgctgcccggccagagcaaaaacttatctctgaagaggacctccaagtgcagctccaacagtctggcgctgagcttgccagaccaggcgcctcagtgaaaatgagttgcaaggccagcggttacaccttcacccgctatacaatgcactgggtgaagcaaagaccgggccagggcctcgaatggatcggctacataaatccatccagggggtacaccaattacaaccagaaattcaaagataaagcaaccctcactaccgacaagagttcaagcacggcttacatgcaactttccagtctgacgtcagaggactccgctgtttactactgcgcacgctactatgatgatcattactcactggattattggggacagggaactacgcttaccgtgtccagcggaggtggtggatcaggaggtggaggttccggaggtggaggaagtggcggtggaggtagcgacatcgtactgactcaatcacccgccattatgagtgcatcaccaggcgagaaagttaccatgacttgttcagcctcatcatctgttagctacatgaattggtatcaacagaagtctgggacctccccaaagagatggatatatgatacctccaaacttgcctctggggtgcctgcacactttagaggaagcggcagcggaaccagctactctctgaccatcagtggaatggaagctgaggacgcagccacctactactgccagcagtggagctctaatccatttacattcggctctggcaccaagcttgaaataaaccgcatagaagtaatgtatccccctccctacttggacaacgagaaatctaacggcacaatcatacacgttaagggcaagcatctgtgtccctcccctcttttccccggaccgtctaagccattttgggtcctcgtggtggtcgggggtgtgctggcctgctacagcttgctggtcacagtggccttcatcatcttctgggtgcgctccaagaggagccggctgcttcacagtgattacatgaacatgacccccaggaggccaggacccaccaggaagcactaccagccctacgctcccccgcgggactttgctgcttaccgcagcagggtcaaattttctagatctgcagatgcgccggcctatcaacaaggccagaaccagctctataacgagctcaatctaggacgaagagaggagtacgatgttttggacaagagacgtggccgggaccctgagatggggggaaagccgagaaggaagaaccctcaggaaggcctgtacaatgaactgcagaaagataagatggcggaggcctacagtgagattgggatgaaaggcgagcgccggaggggcaaggggcacgatggcctttaccagggtctcagtacagccaccaaggacacctacgacgcccttcacatgcaggccctgccccctcgctaaagatctcgagtctagctcgagggcgcgccccgctgatcagcctcgactgtgccttctagttgccagccatctgttgtttgcccctcccccgtgccttccttgaccctggaaggtgccactcccactgtcctttcctaataaaatgaggaaattgcatcgcattgtctgagtaggtgtcattctattctggggggtggggtggggcaggacagcaagggggaggattgggaagacaatagcaggcatgctggggatgcggtgggctctatgggattggtgacagaaaagccccatccttaggcctcctccttcctagtctcctgatattgggtctaacccccacctcctgttaggcagattccttatctggtgacacacccccatttcctggagccatctctctccttgccagaacctctaaggtttgcttacgatggagccagagaggatcctgggagggagagcttggcagggggtgggagggaagggggggatgcgtgacctgcccggttctcagtggccaccctgcgctaccctctcccagaacctgagctgctctgacgcggccgtctggtgcgtttcactgatcctggtgctgcagcttccttacacttcccaagaggagaagcagtttggaaaaacaaaatcagaataagttggtcctgagttct

SEQ ID NO: 16 - DNA, 3229 bp, synthetic construct
  source 1..3229: mol_type = other DNA
accgtttttctggacaaccccaaagtaccccgtctccctggctttagccacctctccatcctcttgctttctttgcctggacaccccgttctcctgtggattcgggtcacctctcactcctttcatttgggcagctcccctaccccccttacctctctagtctgtgctagctcttccagccccctgtcatggcatcttccaggggtccgagagctcagctagtcttcttcctccaacccgggcccctatgtccacttcaggacagcatgtttgctgcctccagggatcctgtgtccccgagctgggaccaccttatattcccagggccggttaatgtggctctggttctgggtacttttatctgtcccctccaccccacagtggggccactagggacagcattgattattgagtagttattaatagtaatcaattacggggtcattagttcatagcccatatatggagttccgcgttacataacttacggtaaatggcccgcctggctgaccgcccaacgacccccgcccattgacgtcaataatgacgtatgttcccatagtaacgccaatagggactttccattgacgtcaatgggtggagtatttacggtaaactgcccacttggcagtacatcaagtgtatcatatgccaagtacgccccctattgacgtcaatgacggtaaatggcccgcctggcattatgcccagtacatgaccttatgggactttcctacttggcagtacatctacgtattagtcatcgctattaccatggtgatgcggttttggcagtacatcaatgggcgtggatagcggtttgactcacggggatttccaagtctccaccccattgacgtcaatgggagtttgttttggcaccaaaatcaacgggactttccaaaatgtcgtaacaactccgccccattgacgcaaatgggcggtaggcgtgtacggtgggaggtctatataagcagagctggtttagtgaaccgtcagatccgctagcgctaccggtcgccaccatggctcttcctgtgactgcccttctgctgcccctggctctcctgctccatgctgcccggccagagcaaaaacttatctctgaagaggacctcgaagtacagctgcagcaaagtggtcccgaattggtgaaacccggtgcatccgtgaaaatgagttgcaaagcatctggctacaaatttacctcctatgtcatgcattgggtgaagcaaaagcccggacaaggcttggagtggatcggctatatcaacccatataacgacgtaacgaaatacaatgaaaaatttaaaggcaaggcgactctgacctcagacaaatctagctctactgcttacatggagctctccagtctgacgagcgaagacagcgccgttcattactgtgcacgaggttcttattatgattacgatggttttgtctattggggacaaggaacgcttgtcactgtatctgctggaggtggtggatcaggaggtggaggttccggaggtggaggaagtggcggtggaggtagccaaattgtgctgacacagagcccggcaatcatgagcgcatctcccggagaaaaggtcaccatgacatgttctgccacctcttctgtctcttacatgcactggtatcagcagaaatcaggcacaagtcctaagagatggatatacgacacaagcaaactggcgagcggagtgcctgctcgcttctccggcagtggaagcgggactagctatagccttaccatcagcagcatggaggccgaagacgccgcaacctactattgtcaacagtggtccagtaaccctctgacttttggagccggaacaaagctggaactcaagttcgtgccagttttcttacccgcgaagccgaccacaacaccagcaccgcgcccaccaacaccagctcccacaatagcctcgcagccgctctcactgcgcccggaggcttgtaggcccgctgccggtggagcagttcatacgcgaggacttgatttcgcctgtgacatatatatttgggcacctctcgccggaacctgtggggtcttgctgctgtctctcgttataacgctttattgcaaacggggcagaaagaaactcctgtatatattcaaacaaccatttatgagaccagtacaaactactcaagaggaagatggctgtagctgccgatttccagaagaagaagaaggaggatgtgaactgagggtcaaattttctagatctgcagatgcgccggcctatcaacaaggccagaaccagctctataacgagctcaatctaggacgaagagaggagtacgatgttttggacaagagacgtggccgggaccctgagatggggggaaagccgagaaggaagaaccctcaggaaggcctgtacaatgaactgcagaaagataagatggcggaggcctacagtgagattgggatgaaaggcgagcgccggaggggcaaggggcacgatggcctttaccagggtctcagtacagccaccaaggacacctacgacgcccttcacatgcaggccctgccccctcgctaaagatctcgagtctagctcgagggcgcgccccgctgatcagcctcgactgtgccttctagttgccagccatctgttgtttgcccctcccccgtgccttccttgaccctggaaggtgccactcccactgtcctttcctaataaaatgaggaaattgcatcgcattgtctgagtaggtgtcattctattctggggggtggggtggggcaggacagcaagggggaggattgggaagacaatagcaggcatgctggggatgcggtgggctctatgggattggtgacagaaaagccccatccttaggcctcctccttcctagtctcctgatattgggtctaacccccacctcctgttaggcagattccttatctggtgacacacccccatttcctggagccatctctctccttgccagaacctctaaggtttgcttacgatggagccagagaggatcctgggagggagagcttggcagggggtgggagggaagggggggatgcgtgacctgcccggttctcagtggccaccctgcgctaccctctcccagaacctgagctgctctgacgcggccgtctggtgcgtttcactgatcctggtgctgcagcttccttacacttcccaagaggagaagcagtttggaaaaacaaaatcagaataagttggtcctgagttct

SEQ ID NO: 17 - DNA, 3229 bp, synthetic construct
  source 1..3229: mol_type = other DNA
accgtttttctggacaaccccaaagtaccccgtctccctggctttagccacctctccatcctcttgctttctttgcctggacaccccgttctcctgtggattcgggtcacctctcactcctttcatttgggcagctcccctaccccccttacctctctagtctgtgctagctcttccagccccctgtcatggcatcttccaggggtccgagagctcagctagtcttcttcctccaacccgggcccctatgtccacttcaggacagcatgtttgctgcctccagggatcctgtgtccccgagctgggaccaccttatattcccagggccggttaatgtggctctggttctgggtacttttatctgtcccctccaccccacagtggggccactagggacagcattgattattgagtagttattaatagtaatcaattacggggtcattagttcatagcccatatatggagttccgcgttacataacttacggtaaatggcccgcctggctgaccgcccaacgacccccgcccattgacgtcaataatgacgtatgttcccatagtaacgccaatagggactttccattgacgtcaatgggtggagtatttacggtaaactgcccacttggcagtacatcaagtgtatcatatgccaagtacgccccctattgacgtcaatgacggtaaatggcccgcctggcattatgcccagtacatgaccttatgggactttcctacttggcagtacatctacgtattagtcatcgctattaccatggtgatgcggttttggcagtacatcaatgggcgtggatagcggtttgactcacggggatttccaagtctccaccccattgacgtcaatgggagtttgttttggcaccaaaatcaacgggactttccaaaatgtcgtaacaactccgccccattgacgcaaatgggcggtaggcgtgtacggtgggaggtctatataagcagagctggtttagtgaaccgtcagatccgctagcgctaccggtcgccaccatggctcttcctgtgactgcccttctgctgcccctggctctcctgctccatgctgcccggccagagcaaaaacttatctctgaagaggacctccaagtgcagctccaacagtctggcgctgagcttgccagaccaggcgcctcagtgaaaatgagttgcaaggccagcggttacaccttcacccgctatacaatgcactgggtgaagcaaagaccgggccagggcctcgaatggatcggctacataaatccatccagggggtacaccaattacaaccagaaattcaaagataaagcaaccctcactaccgacaagagttcaagcacggcttacatgcaactttccagtctgacgtcagaggactccgctgtttactactgcgcacgctactatgatgatcattactcactggattattggggacagggaactacgcttaccgtgtccagcggaggtggtggatcaggaggtggaggttccggaggtggaggaagtggcggtggaggtagcgacatcgtactgactcaatcacccgccattatgagtgcatcaccaggcgagaaagttaccatgacttgttcagcctcatcatctgttagctacatgaattggtatcaacagaagtctgggacctccccaaagagatggatatatgatacctccaaacttgcctctggggtgcctgcacactttagaggaagcggcagcggaaccagctactctctgaccatcagtggaatggaagctgaggacgcagccacctactactgccagcagtggagctctaatccatttacattcggctctggcaccaagcttgaaataaaccgcttcgtgccagttttcttacccgcgaagccgaccacaacaccagcaccgcgcccaccaacaccagctcccacaatagcctcgcagccgctctcactgcgcccggaggcttgtaggcccgctgccggtggagcagttcatacgcgaggacttgatttcgcctgtgacatatatatttgggcacctctcgccggaacctgtggggtcttgctgctgtctctcgttataacgctttattgcaaacggggcagaaagaaactcctgtatatattcaaacaaccatttatgagaccagtacaaactactcaagaggaagatggctgtagctgccgatttccagaagaagaagaaggaggatgtgaactgagggtcaaattttctagatctgcagatgcgccggcctatcaacaaggccagaaccagctctataacgagctcaatctaggacgaagagaggagtacgatgttttggacaagagacgtggccgggaccctgagatggggggaaagccgagaaggaagaaccctcaggaaggcctgtacaatgaactgcagaaagataagatggcggaggcctacagtgagattgggatgaaaggcgagcgccggaggggcaaggggcacgatggcctttaccagggtctcagtacagccaccaaggacacctacgacgcccttcacatgcaggccctgccccctcgctaaagatctcgagtctagctcgagggcgcgccccgctgatcagcctcgactgtgccttctagttgccagccatctgttgtttgcccctcccccgtgccttccttgaccctggaaggtgccactcccactgtcctttcctaataaaatgaggaaattgcatcgcattgtctgagtaggtgtcattctattctggggggtggggtggggcaggacagcaagggggaggattgggaagacaatagcaggcatgctggggatgcggtgggctctatgggattggtgacagaaaagccccatccttaggcctcctccttcctagtctcctgatattgggtctaacccccacctcctgttaggcagattccttatctggtgacacacccccatttcctggagccatctctctccttgccagaacctctaaggtttgcttacgatggagccagagaggatcctgggagggagagcttggcagggggtgggagggaagggggggatgcgtgacctgcccggttctcagtggccaccctgcgctaccctctcccagaacctgagctgctctgacgcggccgtctggtgcgtttcactgatcctggtgctgcagcttccttacacttcccaagaggagaagcagtttggaaaaacaaaatcagaataagttggtcctgagttct

SEQ ID NO: 18 - DNA, 20 bp, synthetic construct
  source 1..20: mol_type = other DNA
ggggccactagggacaggat

SEQ ID NO: 19 - protein, 21 aa, synthetic construct
MALPVTALLLPLALLLHAARP

SEQ ID NO: 20 - protein, 10 aa, synthetic construct
EQKLISEEDL

SEQ ID NO: 21 - protein, 246 aa, synthetic construct
EVQLQQSGPELVKPGASVKMSCKASGYKFTSYVMHWVKQKPGQGLEWIGYINPYNDVTKYNEKFKGKATLTSDKSSSTAYMELSSLTSEDSAVHYCARGSYYDYDGFVYWGQGTLVTVSAGGGGSGGGGSGGGGSGGGGSQIVLTQSPAIMSASPGEKVTMTCSATSSVSYMHWYQQKSGTSPKRWIYDTSKLASGVPARFSGSGSGTSYSLTISSMEAEDAATYYCQQWSSNPLTFGAGTKLELK

SEQ ID NO: 22 - protein, 246 aa, synthetic construct
QVQLQQSGAELARPGASVKMSCKASGYTFTRYTMHWVKQRPGQGLEWIGYINPSRGYTNYNQKFKDKATLTTDKSSSTAYMQLSSLTSEDSAVYYCARYYDDHYSLDYWGQGTTLTVSSGGGGSGGGGSGGGGSGGGGSDIVLTQSPAIMSASPGEKVTMTCSASSSVSYMNWYQQKSGTSPKRWIYDTSKLASGVPAHFRGSGSGTSYSLTISGMEAEDAATYYCQQWSSNPFTFGSGTKLEINR

SEQ ID NO: 23 - protein, 107 aa, synthetic construct
IEVMYPPPYLDNEKSNGTIIHVKGKHLCPSPLFPGPSKPFWVLVVVGGVLACYSLLVTVAFIIFWVRSKRSRLLHSDYMNMTPRRPGPTRKHYQPYAPPRDFAAYRS

SEQ ID NO: 24 - protein, 79 aa, synthetic construct
FVPVFLPAKPTTTPAPRPPTPAPTIASQPLSLRPEACRPAAGGAVHTRGLDFACDIYIWAPLAGTCGVLLLSLVITLYC

SEQ ID NO: 25 - protein, 42 aa, synthetic construct
KRGRKKLLYIFKQPFMRPVQTTQEEDGCSCRFPEEEEGGCEL

SEQ ID NO: 26 - protein, 112 aa, synthetic construct
RVKFSRSADAPAYQQGQNQLYNELNLGRREEYDVLDKRRGRDPEMGGKPRRKNPQEGLYNELQKDKMAEAYSEIGMKGERRRGKGHDGLYQGLSTATKDTYDALHMQALPPR

SEQ ID NO: 27 - protein, 496 aa, synthetic construct
MALPVTALLLPLALLLHAARPEQKLISEEDLEVQLQQSGPELVKPGASVKMSCKASGYKFTSYVMHWVKQKPGQGLEWIGYINPYNDVTKYNEKFKGKATLTSDKSSSTAYMELSSLTSEDSAVHYCARGSYYDYDGFVYWGQGTLVTVSAGGGGSGGGGSGGGGSGGGGSQIVLTQSPAIMSASPGEKVTMTCSATSSVSYMHWYQQKSGTSPKRWIYDTSKLASGVPARFSGSGSGTSYSLTISSMEAEDAATYYCQQWSSNPLTFGAGTKLELKIEVMYPPPYLDNEKSNGTIIHVKGKHLCPSPLFPGPSKPFWVLVVVGGVLACYSLLVTVAFIIFWVRSKRSRLLHSDYMNMTPRRPGPTRKHYQPYAPPRDFAAYRSRVKFSRSADAPAYQQGQNQLYNELNLGRREEYDVLDKRRGRDPEMGGKPRRKNPQEGLYNELQKDKMAEAYSEIGMKGERRRGKGHDGLYQGLSTATKDTYDALHMQALPPR

SEQ ID NO: 28 - protein, 496 aa, synthetic construct
MALPVTALLLPLALLLHAARPEQKLISEEDLQVQLQQSGAELARPGASVKMSCKASGYTFTRYTMHWVKQRPGQGLEWIGYINPSRGYTNYNQKFKDKATLTTDKSSSTAYMQLSSLTSEDSAVYYCARYYDDHYSLDYWGQGTTLTVSSGGGGSGGGGSGGGGSGGGGSDIVLTQSPAIMSASPGEKVTMTCSASSSVSYMNWYQQKSGTSPKRWIYDTSKLASGVPAHFRGSGSGTSYSLTISGMEAEDAATYYCQQWSSNPFTFGSGTKLEINRIEVMYPPPYLDNEKSNGTIIHVKGKHLCPSPLFPGPSKPFWVLVVVGGVLACYSLLVTVAFIIFWVRSKRSRLLHSDYMNMTPRRPGPTRKHYQPYAPPRDFAAYRSRVKFSRSADAPAYQQGQNQLYNELNLGRREEYDVLDKRRGRDPEMGGKPRRKNPQEGLYNELQKDKMAEAYSEIGMKGERRRGKGHDGLYQGLSTATKDTYDALHMQALPPR

SEQ ID NO: 29 - protein, 510 aa, synthetic construct
MALPVTALLLPLALLLHAARPEQKLISEEDLEVQLQQSGPELVKPGASVKMSCKASGYKFTSYVMHWVKQKPGQGLEWIGYINPYNDVTKYNEKFKGKATLTSDKSSSTAYMELSSLTSEDSAVHYCARGSYYDYDGFVYWGQGTLVTVSAGGGGSGGGGSGGGGSGGGGSQIVLTQSPAIMSASPGEKVTMTCSATSSVSYMHWYQQKSGTSPKRWIYDTSKLASGVPARFSGSGSGTSYSLTISSMEAEDAATYYCQQWSSNPLTFGAGTKLELKFVPVFLPAKPTTTPAPRPPTPAPTIASQPLSLRPEACRPAAGGAVHTRGLDFACDIYIWAPLAGTCGVLLLSLVITLYCKRGRKKLLYIFKQPFMRPVQTTQEEDGCSCRFPEEEEGGCELRVKFSRSADAPAYQQGQNQLYNELNLGRREEYDVLDKRRGRDPEMGGKPRRKNPQEGLYNELQKDKMAEAYSEIGMKGERRRGKGHDGLYQGLSTATKDTYDALHMQALPPR

SEQ ID NO: 30 - protein, 510 aa, synthetic construct
MALPVTALLLPLALLLHAARPEQKLISEEDLQVQLQQSGAELARPGASVKMSCKASGYTFTRYTMHWVKQRPGQGLEWIGYINPSRGYTNYNQKFKDKATLTTDKSSSTAYMQLSSLTSEDSAVYYCARYYDDHYSLDYWGQGTTLTVSSGGGGSGGGGSGGGGSGGGGSDIVLTQSPAIMSASPGEKVTMTCSASSSVSYMNWYQQKSGTSPKRWIYDTSKLASGVPAHFRGSGSGTSYSLTISGMEAEDAATYYCQQWSSNPFTFGSGTKLEINRFVPVFLPAKPTTTPAPRPPTPAPTIASQPLSLRPEACRPAAGGAVHTRGLDFACDIYIWAPLAGTCGVLLLSLVITLYCKRGRKKLLYIFKQPFMRPVQTTQEEDGCSCRFPEEEEGGCELRVKFSRSADAPAYQQGQNQLYNELNLGRREEYDVLDKRRGRDPEMGGKPRRKNPQEGLYNELQKDKMAEAYSEIGMKGERRRGKGHDGLYQGLSTATKDTYDALHMQALPPR

SEQ ID NO: 31 - protein, 121 aa, synthetic construct
EVQLQQSGPELVKPGASVKMSCKASGYKFTSYVMHWVKQKPGQGLEWIGYINPYNDVTKYNEKFKGKATLTSDKSSSTAYMELSSLTSEDSAVHYCARGSYYDYDGFVYWGQGTLVTVSAG

SEQ ID NO: 32 - protein, 106 aa, synthetic construct
QIVLTQSPAIMSASPGEKVTMTCSATSSVSYMHWYQQKSGTSPKRWIYDTSKLASGVPARFSGSGSGTSYSLTISSMEAEDAATYYCQQWSSNPLTFGAGTKLELK

SEQ ID NO: 33 - protein, 5 aa, synthetic construct
SYVMH

SEQ ID NO: 34 - protein, 17 aa, synthetic construct
YINPYNDVTKYNEKFKG

SEQ ID NO: 35 - protein, 11 aa, synthetic construct
GSYYDYDGFVY

SEQ ID NO: 36 - protein, 10 aa, synthetic construct
SATSSVSYMH

SEQ ID NO: 37 - protein, 7 aa, synthetic construct
DTSKLAS

SEQ ID NO: 38 - protein, 9 aa, synthetic construct
QQWSSNPLT

SEQ ID NO: 39 - protein, 120 aa, synthetic construct
QVQLQQSGAELARPGASVKMSCKASGYTFTRYTMHWVKQRPGQGLEWIGYINPSRGYTNYNQKFKDKATLTTDKSSSTAYMQLSSLTSEDSAVYYCARYYDDHYSLDYWGQGTTLTVSSG

SEQ ID NO: 40 - protein, 106 aa, synthetic construct
DIVLTQSPAIMSASPGEKVTMTCSASSSVSYMNWYQQKSGTSPKRWIYDTSKLASGVPAHFRGSGSGTSYSLTISGMEAEDAATYYCQQWSSNPFTFGSGTKLEIN

SEQ ID NO: 41 - protein, 5 aa, synthetic construct
RYTMH

SEQ ID NO: 42 - protein, 17 aa, synthetic construct
YINPSRGYTNYNQKFKD

SEQ ID NO: 43 - protein, 10 aa, synthetic construct
YYDDHYSLDY

SEQ ID NO: 44 - protein, 10 aa, synthetic construct
SASSSVSYMN

SEQ ID NO: 45 - protein, 7 aa, synthetic construct
DTSKLAS

SEQ ID NO: 46 - protein, 9 aa, synthetic construct
QQWSSNPFT

SEQ ID NO: 47 - protein, 19 aa, synthetic construct
GGGSGGGGSGGGGSGGGGS

SEQ ID NO: 48 - protein, 18 aa, synthetic construct
GSTSGSGKPGSGEGSTKG

SEQ ID NO: 49 - protein, 237 aa, synthetic construct
PAEPKSPDKTHTCPPCPAPPVAGPSVFLFPPKPKDTLMIARTPEVTCVVVDVSHEDPEVKFNWYVDGVEVHNAKTKPREEQYNSTYRVVSVLTVLHQDWLNGKEYKCKVSNKALPAPIEKTISKAKGQPREPQVYTLPPSRDELTKNQVSLTCLVKGFYPSDIAVEWESNGQPENNYKTTPPVLDSDGSFFLYSKLTVDKSRWQQGNVFSCSVMHEALHNHYTQKSLSLSPGKKDPK

SEQ ID NO: 50 - protein, 235 aa, synthetic construct
PAEPKSPDKTHTCPPCPAPPVAGPSVFLFPPKPKDTLMIARTPEVTCVVVDVSHEDPEVKFNWYVDGVEVHNAKTKPREEQYNSTYRVVSVLTVLHQDWLNGKEYKCKVSNKALPAPIEKTISKAKGQPREPQVYTLPPSRDELTKNQVSLTCLVKGFYPSDIAVEWESNGQPENNYKTTPPVLDSDGSFFLYSKLTVDKSRWQQGNVFSCSVMHEALHNHYTQKSLSSLSPGKK

SEQ ID NO: 51 - protein, 229 aa, synthetic construct
ESKYGPPCPPCPAPEFEGGPSVFLFPPKPKDTLMISRTPEVTCVVVDVSQEDPEVQFNWYVDGVEVHNAKTKPREEQFNSTYRVVSVLTVLHQDWLNGKEYKCKVSNKGLPSSIEKTISKAKGQPREPQVYTLPPSQEEMTKNQVSLTCLVKGFYPSDIAVEWESNGQPENNYKTTPPVLDSDGSFFLYSRLTVDKSRWQEGNVFSCSVMHEALHNHYTQKSLSLSLGK

SEQ ID NO: 52 - protein, 119 aa, synthetic construct
ESKYGPPCPPCPGQPREPQVYTLPPSQEEMTKNQVSLTCLVKGFYPSDIAVEWESNGQPENNYKTTPPVLDSDGSFFLYSRLTVDKSRWQEGNVFSCSVMHEALHNHYTQKSLSLSLGK

SEQ ID NO: 53 - protein, 12 aa, synthetic construct
ESKYGPPCPPCP